European Patent Application EP 4 807 007 A1, published September 16, 2026. Title: 一种含有双噬菌体来源启动子的组成型表达载体、包含其的细菌及应用. Applicant: 上海缮维特生物技术有限公司. The sequence listing filed with the application follows.

SEQUENCE LISTING (101 sequences)

SEQ ID NO: 1 - DNA, 18 bp, Artificial sequence
  source 1..18: mol_type = other DNA
taatacgactcactatag

SEQ ID NO: 2 - DNA, 18 bp, Artificial sequence
  source 1..18: mol_type = other DNA
aattaaccctcactaaag

SEQ ID NO: 3 - DNA, 18 bp, Artificial sequence
  source 1..18: mol_type = other DNA
atttaggtgacactatag

SEQ ID NO: 4 - DNA, 2652 bp, Artificial sequence
  source 1..2652: mol_type = other DNA
atgaacaccatcaacattgccaaaaacgattttagcgatattgaactggcagcgattccgtttaataccctggcagatcattatggtgaacgtctggcacgtgaacagctggcactggaacatgaaagctatgaaatgggtgaagcacgttttcgcaaaatgtttgaacgtcagctgaaagccggtgaagttgcagataatgcagcagcaaaaccgctgattaccacactgctgccgaaaatgattgcacgtattaacgattggttcgaagaggttaaagccaaacgtggtaaacgtccgaccgcatttcagtttctgcaagaaattaaaccggaagccgttgcctatattaccattaaaaccacactggcatgtctgaccagcgcagataataccaccgttcaggcagttgcaagcgcaattggtcgtgcaattgaagatgaagcccgttttggtcgtattcgtgatctggaagcaaaacactttaagaaaaacgtggaagaacagctgaataaacgtgttggtcacgtttataagaaagcctttatgcaggttgttgaagcagatatgctgagcaaaggtctgttaggtggtgaagcatggtcaagctggcataaagaagatagcattcacgttggtgttcgctgtattgaaatgctgattgaaagcaccggtatggttagcctgcatcgtcagaatgccggtgttgttggtcaggatagcgaaaccatcgaactggcaccggaatatgccgaagcaattgcaacccgtgccggtgcactggcaggtattagcccgatgtttcagccgtgtgttgttccgcctaaaccgtggaccggcattaccggtggtggttattgggcaaatggtcgtcgtccgctggcgctggttcgtacccatagcaaaaaggcactgatgcgttatgaagatgtttatatgccggaagtgtacaaagccattaacattgcacagaataccgcctggaaaatcaataaaaaggttctggccgttgccaacgttatcaccaaatggaaacattgtccggttgaagatattccggcaattgaacgtgaagaactgccgatgaagccggaagatattgatatgaatccggaagcactgaccgcatggaaacgtgcagcagccgcagtttatcgtaaagataaagcacgtaaaagccgtcgtattagcctggaatttatgctggaacaggcaaacaaatttgccaaccataaagcaatctggttcccgtataatatggattggcgtggtcgtgtttatgccgttagcatgtttaatccgcagggtaatgatatgaccaaaggcctgctgaccctggcaaaaggtaaaccgattggtaaagaaggttactattggctgaaaattcatggtgcaaattgtgccggtgtggataaagttccgtttccggaacgcattaaattcatcgaagaaaaccacgaaaacattatggcctgtgcaaaaagtccgctggaaaatacctggtgggcagaacaggatagtccgttttgttttctggccttttgttttgaatatgcgggtgttcagcatcatggtctgagctataattgtagcctgccgctggcatttgatggtagctgtagcggtattcagcattttagcgcaatgctgcgtgatgaagttggtggtcgtgccgttaatctgctgccgtcagaaaccgtgcaggatatttatggtattgttgccaagaaagtgaacgaaattctgcaagcagatgcaattaatggcaccgataatgaagttgttaccgtgaccgatgaaaacaccggtgaaattagcgaaaaagttaaactgggcaccaaagcgctggcaggtcagtggctggcctatggtgttacccgtagcgttaccaaacgtagcgtgatgacactggcgtatggtagcaaagaatttggttttcgtcagcaggttctggaagatacaattcagcctgcaattgatagcggtaaaggtctgatgtttacccagccgaatcaggcagcaggttatatggcaaaactgatttgggaaagcgttagcgtgaccgttgttgcagcagttgaagcaatgaactggctgaaatcagcagccaaactgctggcagcagaagttaaagataagaaaacgggtgaaatcctgcgtaaacgttgtgccgttcattgggttacaccggatggttttccggtttggcaagaatataagaaaccgattcagacacgcctgaacctgatgtttctgggtcagtttcgtctgcaaccgaccattaataccaataaagattccgaaatcgacgcccacaaacaagaaagcggtattgcaccgaattttgttcatagccaggatggtagccatctgcgtaaaaccgttgtttgggcacatgaaaaatatggcattgaatcctttgcgctgatccatgatagctttggcaccattccggcagatgcagcaaacctgtttaaagcagttcgtgaaacaatggtggatacctatgaaagctgtgatgttctggcggatttttatgatcagtttgcagatcagctgcatgaaagccagctggataaaatgcctgcactgcctgccaaaggtaatctgaatctgcgtgatattctggaaagcgattttgcctttgcctaa

SEQ ID NO: 5 - protein, 883 aa, Artificial sequence
MNTINIAKNDFSDIELAAIPFNTLADHYGERLAREQLALEHESYEMGEARFRKMFERQLKAGEVADNAAAKPLITTLLPKMIARINDWFEEVKAKRGKRPTAFQFLQEIKPEAVAYITIKTTLACLTSADNTTVQAVASAIGRAIEDEARFGRIRDLEAKHFKKNVEEQLNKRVGHVYKKAFMQVVEADMLSKGLLGGEAWSSWHKEDSIHVGVRCIEMLIESTGMVSLHRQNAGVVGQDSETIELAPEYAEAIATRAGALAGISPMFQPCVVPPKPWTGITGGGYWANGRRPLALVRTHSKKALMRYEDVYMPEVYKAINIAQNTAWKINKKVLAVANVITKWKHCPVEDIPAIEREELPMKPEDIDMNPEALTAWKRAAAAVYRKDKARKSRRISLEFMLEQANKFANHKAIWFPYNMDWRGRVYAVSMFNPQGNDMTKGLLTLAKGKPIGKEGYYWLKIHGANCAGVDKVPFPERIKFIEENHENIMACAKSPLENTWWAEQDSPFCFLAFCFEYAGVQHHGLSYNCSLPLAFDGSCSGIQHFSAMLRDEVGGRAVNLLPSETVQDIYGIVAKKVNEILQADAINGTDNEVVTVTDENTGEISEKVKLGTKALAGQWLAYGVTRSVTKRSVMTLAYGSKEFGFRQQVLEDTIQPAIDSGKGLMFTQPNQAAGYMAKLIWESVSVTVVAAVEAMNWLKSAAKLLAAEVKDKKTGEILRKRCAVHWVTPDGFPVWQEYKKPIQTRLNLMFLGQFRLQPTINTNKDSEIDAHKQESGIAPNFVHSQDGSHLRKTVVWAHEKYGIESFALIHDSFGTIPADAANLFKAVRETMVDTYESCDVLADFYDQFADQLHESQLDKMPALPAKGNLNLRDILESDFAFA

SEQ ID NO: 6 - DNA, 2655 bp, Artificial sequence
  source 1..2655: mol_type = other DNA
atgaacatcatcgaaaacatcgaaaagaatgacttctcagaaatcgaactggctgctatcccgttcaacacactggctgaccactacggaagcgccttggctaaagagcagttggctttagaacatgagtcttatgagctaggcgagcgccgcttcctcaagatgcttgagcgtcaagcgaaagctggtgagattgcagacaacgcagccgctaagccgttactcgctacgcttctccctaagttaaccacacgtatcgtcgagtggctcgaagagtacgcatcgaagaaaggccgcaagcctagcgcatacgcaccgctccagttactcaagccggaggcctccgcgtttatcaccctgaaagttatccttgcgtcactaaccagtacgaacatgacaaccattcaggccgctgctggtatgctggggaaagccattgaggacgaggcacgatttgggcgcatccgtgacctagaagcgaagcacttcaagaagcacgttgaggaacagcttaacaagcgccacgggcaagtctacaagaaagcatttatgcaggtggtcgaggccgatatgattggtcgaggtctgcttggtggcgaggcgtggtctagctgggataaagaaaccacgatgcacgtagggattcgcctgattgaaatgctgattgaatccacgggtctggtggaattacagcgccacaacgcaggtaacgcaggctctgaccatgaggcactgcaactggcccaagagtacgtggacgtattagcgaagcgtgcaggcgctctggcgggtatctctccgatgttccagccgtgtgtcgtaccgccgaaaccttgggtagcaatcacagggggcggctattgggctaacggtcgcagacctttggcactcgttcgcactcactctaagaagggcttgatgcgctacgaagacgtttacatgccagaagtctacaaggctgtgaacctcgcgcaaaacaccgcatggaaaatcaacaagaaagttcttgctgttgtcaatgagattgttaactggaagaattgcccggtagcagacattccatcgctggagcgccaagagttaccgcctaagcctgacgacattgacaccaacgaggcagcgctcaaggagtggaagaaagccgctgctggtatctatcgcttggacaaggcacgagtgtctcgccgtatcagcttagagttcatgctggagcaggccaacaagttcgcaagtaagaaagcaatctggttcccttacaacatggactggcgcggtcgtgtgtacgctgtgccgatgttcaacccgcaaggcaacgacatgacgaaaggtctgctgacccttgctaaaggcaagccaatcggtgaggaaggtttctactggctgaaaatccacggtgcgaactgtgcgggtgttgataaggttccattcccggagcgcatcgcgttcattgagaagcacgtagacgacattctggcttgcgctaaagacccaatcaataacacttggtgggctgagcaggattcaccgttctgtttcctcgcgttttgcttcgagtatgcaggcgttacgcaccacggtctgagctacaattgctctctgccgctggcgttcgacgggtcttgctctggtatccagcacttctccgcgatgctccgcgatgaggtaggcggtcgtgcggttaacctgctgccaagcgaaaccgtgcaggacatttacggcatcgttgcacagaaagtaaacgagattctcaaacaggatgcaatcaacggcacgcctaacgagatgattaccgtgaccgacaaggacaccggggaaatctcagagaagctcaaacttggaacctcaacgctggcgcaacagtggctggcatatggtgtaacccgtagcgtaactaaacgttcggtcatgacgctggcttacggttccaaggagttcggctttcgtcaacaggtattggatgacaccattcagcctgcaattgacagcggtaagggcttgatgttcacccaaccgaaccaagcggctggctatatggctaagctgatttgggatgcggtaagcgtgaccgtagttgcagcggttgaggcgatgaactggctcaaatctgccgctaagctgctggctgctgaggtcaaggacaagaagaccaaggagattctgcgccaccgttgcgcggttcactggactacgccggacggcttcccggtctggcaggaataccgcaagccactccagaagcgtctcgatatgattttcttagggcaattccgtctgcaaccgacgattaataccctcaaggattcaggcattgacgcacacaagcaggagtctggcatcgctcctaactttgttcactcacaggacggtagccacctccgcatgacagtcgtttatgctcacgagaagtatggcattgagtcctttgcgctcatccatgacagctttgggactatcccggcagacgctggtaagctctttaaggctgtgcgtgaaacgatggttatcacctatgagaacaacgatgtgctggcagacttctactctcagtttgccgaccagctacacgagacccaactggacaagatgcctccgcttccgaagaaaggaaacctgaacctgcaagacattctcaagtctgactttgcctttgcataa

SEQ ID NO: 7 - protein, 884 aa, Artificial sequence
MNIIENIEKNDFSEIELAAIPFNTLADHYGSALAKEQLALEHESYELGERRFLKMLERQAKAGEIADNAAAKPLLATLLPKLTTRIVEWLEEYASKKGRKPSAYAPLQLLKPEASAFITLKVILASLTSTNMTTIQAAAGMLGKAIEDEARFGRIRDLEAKHFKKHVEEQLNKRHGQVYKKAFMQVVEADMIGRGLLGGEAWSSWDKETTMHVGIRLIEMLIESTGLVELQRHNAGNAGSDHEALQLAQEYVDVLAKRAGALAGISPMFQPCVVPPKPWVAITGGGYWANGRRPLALVRTHSKKGLMRYEDVYMPEVYKAVNLAQNTAWKINKKVLAVVNEIVNWKNCPVADIPSLERQELPPKPDDIDTNEAALKEWKKAAAGIYRLDKARVSRRISLEFMLEQANKFASKKAIWFPYNMDWRGRVYAVPMFNPQGNDMTKGLLTLAKGKPIGEEGFYWLKIHGANCAGVDKVPFPERIAFIEKHVDDILACAKDPINNTWWAEQDSPFCFLAFCFEYAGVTHHGLSYNCSLPLAFDGSCSGIQHFSAMLRDEVGGRAVNLLPSETVQDIYGIVAQKVNEILKQDAINGTPNEMITVTDKDTGEISEKLKLGTSTLAQQWLAYGVTRSVTKRSVMTLAYGSKEFGFRQQVLDDTIQPAIDSGKGLMFTQPNQAAGYMAKLIWDAVSVTVVAAVEAMNWLKSAAKLLAAEVKDKKTKEILRHRCAVHWTTPDGFPVWQEYRKPLQKRLDMIFLGQFRLQPTINTLKDSGIDAHKQESGIAPNFVHSQDGSHLRMTVVYAHEKYGIESFALIHDSFGTIPADAGKLFKAVRETMVITYENNDVLADFYSQFADQLHETQLDKMPPLPKKGNLNLQDILKSDFAFA

SEQ ID NO: 8 - DNA, 2625 bp, Artificial sequence
  source 1..2625: mol_type = other DNA
atgcaagatttacacgctatccagcttcaattagaagaagagatgtttaatggtggcattcgtcgcttcgaagcagatcaacaacgccagattgcagcaggtagcgagagcgacacagcatggaaccgccgcctgttgtcagaacttattgcacctatggctgaaggcattcaggcttataaagaagagtacgaaggtaagaaaggtcgtgcacctcgcgcattggctttcttacaatgtgtagaaaatgaagttgcagcatacatcactatgaaagttgttatggatatgctgaatacggatgctacccttcaggctattgcaatgagtgtagcagaacgcattgaagaccaagtgcgcttttctaagctagaaggtcacgccgctaaatactttgagaaggttaagaagtcactcaaggctagccgtactaagtcatatcgtcacgctcataacgtagctgtagttgctgaaaaatcagttgcagaaaaggacgcggactttgaccgttgggaggcgtggccaaaagaaactcaattgcagattggtactaccttgcttgaaatcttagaaggtagcgttttctataatggtgaacctgtatttatgcgtgctatgcgcacttatggcggaaagactatttactacttacaaacttctgaaagtgtaggccagtggattagcgcattcaaagagcacgtagcgcaattaagcccagcttatgccccttgcgtaatccctcctcgtccttggagaactccatttaatggagggttccatactgagaaggtagctagccgtatccgtcttgtaaaaggtaaccgtgagcatgtacgcaagttgactcaaaagcaaatgccaaaggtttataaggctatcaacgcattacaaaatacacaatggcaaatcaacaaggatgtattagcagttattgaagaagtaatccgcttagaccttggttatggtgtaccttccttcaagccactgattgacaaggagaacaagccagctaacccggtacctgttgaattccaacacctgcgcggtcgtgaactgaaagagatgctatcacctgagcagtggcaacaattcattaactggaaaggcgaatgcgcgcgcctatataccgcagaaactaagcgcggttcaaagtccgccgccgttgttcgcatggtaggacaggcccgtaaatatagcgcctttgaatccatttacttcgtgtacgcaatggatagccgcagccgtgtctatgtgcaatctagcacgctctctccgcagtctaacgacttaggtaaggcattactccgctttaccgagggacgccctgtgaatggcgtagaagcgcttaaatggttctgcatcaatggtgctaacctttggggatgggacaagaaaacttttgatgtgcgcgtgtctaacgtattagatgaggaattccaagatatgtgtcgagacatcgccgcagaccctctcacattcacccaatgggctaaagctgatgcaccttatgaattcctcgcttggtgctttgagtatgctcaataccttgatttggtggatgaaggaagggccgacgaattccgcactcacctaccagtacatcaggacgggtcttgttcaggcattcagcactatagtgctatgcttcgcgacgaagtaggggccaaagctgttaacctgaaaccctccgatgcaccgcaggatatctatggggcggtggcgcaagtggttatcaagaagaatgcgctatatatggatgcggacgatgcaaccacgtttacttctggtagcgtcacgctgtccggtacagaactgcgagcaatggctagcgcatgggatagtattggtattacccgtagcttaaccaaaaagcccgtgatgaccttgccatatggttctactcgcttaacttgccgtgaatctgtgattgattacatcgtagacttagaggaaaaagaggcgcagaaggcagtagcagaagggcggacggcaaacaaggtacatccttttgaagacgatcgtcaagattacttgactccgggcgcagcttacaactacatgacggcactaatctggccttctatttctgaagtagttaaggcaccgatagtagctatgaagatgatacgccagcttgcacgctttgcagcgaaacgtaatgaaggcctgatgtacaccctgcctactggcttcatcttagaacagaagatcatggcaaccgagatgctacgcgtgcgtacctgtctgatgggtgatatcaagatgtcccttcaggttgaaacggatatcgtagatgaagccgctatgatgggagcagcagcacctaatttcgtacacggtcatgacgcaagtcaccttatccttaccgtatgtgaattggtagacaagggcgtaactagtatcgctgtaatccacgactcttttggtactcatgcagacaacaccctcactcttagagtggcacttaaagggcagatggttgcaatgtatattgatggtaatgcgcttcagaaactactggaggagcatgaagagcgctggatggttgatacaggtatcgaagtacctgagcaaggggagttcgaccttaacgaaatcatggattctgaatacgtatttgcctaa

SEQ ID NO: 9 - protein, 874 aa, Artificial sequence
MQDLHAIQLQLEEEMFNGGIRRFEADQQRQIAAGSESDTAWNRRLLSELIAPMAEGIQAYKEEYEGKKGRAPRALAFLQCVENEVAAYITMKVVMDMLNTDATLQAIAMSVAERIEDQVRFSKLEGHAAKYFEKVKKSLKASRTKSYRHAHNVAVVAEKSVAEKDADFDRWEAWPKETQLQIGTTLLEILEGSVFYNGEPVFMRAMRTYGGKTIYYLQTSESVGQWISAFKEHVAQLSPAYAPCVIPPRPWRTPFNGGFHTEKVASRIRLVKGNREHVRKLTQKQMPKVYKAINALQNTQWQINKDVLAVIEEVIRLDLGYGVPSFKPLIDKENKPANPVPVEFQHLRGRELKEMLSPEQWQQFINWKGECARLYTAETKRGSKSAAVVRMVGQARKYSAFESIYFVYAMDSRSRVYVQSSTLSPQSNDLGKALLRFTEGRPVNGVEALKWFCINGANLWGWDKKTFDVRVSNVLDEEFQDMCRDIAADPLTFTQWAKADAPYEFLAWCFEYAQYLDLVDEGRADEFRTHLPVHQDGSCSGIQHYSAMLRDEVGAKAVNLKPSDAPQDIYGAVAQVVIKKNALYMDADDATTFTSGSVTLSGTELRAMASAWDSIGITRSLTKKPVMTLPYGSTRLTCRESVIDYIVDLEEKEAQKAVAEGRTANKVHPFEDDRQDYLTPGAAYNYMTALIWPSISEVVKAPIVAMKMIRQLARFAAKRNEGLMYTLPTGFILEQKIMATEMLRVRTCLMGDIKMSLQVETDIVDEAAMMGAAAPNFVHGHDASHLILTVCELVDKGVTSIAVIHDSFGTHADNTLTLRVALKGQMVAMYIDGNALQKLLEEHEERWMVDTGIEVPEQGEFDLNEIMDSEYVFA

SEQ ID NO: 10 - DNA, 60 bp, Artificial sequence
  source 1..60: mol_type = other DNA
tcactcattaggcaccccaggctttacactttatgcttccggctcgtataatgtgtggaa

SEQ ID NO: 11 - DNA, 1125 bp, Artificial sequence
  source 1..1125: mol_type = other DNA
ttgcaggaaaaaaacgctatgaaaaatgttggttttatcggctggcgcggaatggtcggctctgttctcatgcaacgcatggtagaggagcgcgatttcgacgctattcgccctgttttcttttctacctcccagtttggacaggcggcgcccaccttcggcgacacctccaccggcacgctacaggacgcttttgatctggatgcgctaaaagcgctcgatatcatcgtgacctgccagggcggcgattataccaacgaaatttatccaaagctgcgcgaaagcggatggcagggttactggattgatgcggcttctacgctgcgcatgaaagatgatgccattattattctcgacccggtcaaccaggacgtgattaccgacggcctgaacaatggcgtgaagacctttgtgggcggtaactgtaccgttagcctgatgttgatgtcgctgggcggtctctttgcccataatctcgttgactgggtatccgtcgcgacctatcaggccgcctccggcggcggcgcgcgccatatgcgcgagctgttaacccagatgggtcagttgtatggccatgtcgccgatgaactggcgacgccgtcttccgcaattcttgatattgaacgcaaagttacggcattgacccgcagcggcgagctgccggttgataactttggcgtaccgctggcgggaagcctgatcccctggatcgacaaacagctcgataacggccagagccgcgaagagtggaaaggccaggcggaaaccaacaagattctcaatactgcctctgtgattccggttgatggtttgtgtgtgcgcgtcggcgcgctgcgctgtcacagccaggcgttcaccatcaagctgaaaaaagaggtatccattccgacggtggaagaactgctggcggcacataatccgtgggcgaaagtggtgccgaacgatcgtgatatcactatgcgcgaattaaccccggcggcggtgaccggcacgttgactacgccggttggtcgtctgcgtaagctgaacatggggccagagttcttgtcggcgtttaccgtaggcgaccagttgttatggggcgccgccgagccgctgcgtcgaatgctgcgccagttggcgtag

SEQ ID NO: 12 - protein, 374 aa, Artificial sequence
LQEKNAMKNVGFIGWRGMVGSVLMQRMVEERDFDAIRPVFFSTSQFGQAAPTFGDTSTGTLQDAFDLDALKALDIIVTCQGGDYTNEIYPKLRESGWQGYWIDAASTLRMKDDAIIILDPVNQDVITDGLNNGVKTFVGGNCTVSLMLMSLGGLFAHNLVDWVSVATYQAASGGGARHMRELLTQMGQLYGHVADELATPSSAILDIERKVTALTRSGELPVDNFGVPLAGSLIPWIDKQLDNGQSREEWKGQAETNKILNTASVIPVDGLCVRVGALRCHSQAFTIKLKKEVSIPTVEELLAAHNPWAKVVPNDRDITMRELTPAAVTGTLTTPVGRLRKLNMGPEFLSAFTVGDQLLWGAAEPLRRMLRQLA

SEQ ID NO: 13 - DNA, 1593 bp, Artificial sequence
  source 1..1593: mol_type = other DNA
atgaaaaaaatcatgctggttttcatcaccctcatactggtaagcctgccgatcgcgcagcagaccgaagcgaaagacgcgtctgcgttcaacaaagaaaactctatctcttctatggcgccgccggcgtctccgccggcgtctccgaaaaccccgatcgaaaaaaaacacgcggacgaaatcgacaaatacatccagggcctggactacaacaaaaacaacgttctggtttaccacggcgacgcggttaccaacgttccgccgcgtaaaggctacaaagacggcaacgaatacatcgttgttgaaaaaaaaaaaaaatctatcaaccagaacaacgcggacatccaggttgttaacgcgatctcttctctgacctacccgggcgcgctggttaaagcgaactctgaactggttgaaaaccagccggacgttctgccggttaaacgtgactctctgaccctgtctatcgacctgccgggcatgaccaaccaggacaacaaaatcgttgttaaaaacgcgaccaaatctaacgttaacaacgcggttaacaccctggttgaacgttggaacgaaaaatacgcgcaggcgtacccgaacgtttctgcgaaaatcgactacgacgacgaaatggcgtactctgaatctcagctgatcgcgaaattcggcaccgcgttcaaagcggttaacaactctctgaacgttaacttcggcgcgatctctgaaggcaaaatgcaggaagaagttatctctttcaaacagatctactacaacgttaacgttaacgaaccgacccgtccgtctcgtttcttcggcaaagcggttaccaaagaacagcttcaggcgctgggcgttaacgcggaaaacccgccggcgtacatctcttctgttgcgtacggccgtcaggtttacctgaaactgtctaccaactctcactctaccaaagttaaagcggctttcgacgcggcggtaagcggcaaatctgtttctggcgacgttgaactgaccaacatcatcaaaaactcttctttcaaagcggttatctacggcggctctgcgaaagacgaagttcagatcatcgacggcaacctgggcgacctgcgtgacatcctgaaaaaaggcgcgaccttcaaccgtgaaaccccgggcgttccgatcgcgtacaccaccaacttcctgaaagacaacgaactggcggttatcaaaaacaactctgaatacatcgaaaccacctctaaagcgtacaccgacggcaaaatcaacatcgaccactctggcggctacgttgcgcagttcaacatctcttgggacgaagttaactacgacccggaaggcaacgaaatcgttcagcacaaaaactggtctgaaaacaacaaatctaaactggcgcacttcacctcttctatctacctgccgggcaacgcgcgtaacatcaacgtttacgcgaaagaatgcaccggcctggcgtgggaatggtggcgtaccgttatcgacgaccgtaacctgccgctggttaaaaaccgtaacatctctatctggggcaccaccctgtacccgaaatactctaacaaagttgacaacccgatcgaataatga

SEQ ID NO: 14 - protein, 529 aa, Artificial sequence
MKKIMLVFITLILVSLPIAQQTEAKDASAFNKENSISSMAPPASPPASPKTPIEKKHADEIDKYIQGLDYNKNNVLVYHGDAVTNVPPRKGYKDGNEYIVVEKKKKSINQNNADIQVVNAISSLTYPGALVKANSELVENQPDVLPVKRDSLTLSIDLPGMTNQDNKIVVKNATKSNVNNAVNTLVERWNEKYAQAYPNVSAKIDYDDEMAYSESQLIAKFGTAFKAVNNSLNVNFGAISEGKMQEEVISFKQIYYNVNVNEPTRPSRFFGKAVTKEQLQALGVNAENPPAYISSVAYGRQVYLKLSTNSHSTKVKAAFDAAVSGKSVSGDVELTNIIKNSSFKAVIYGGSAKDEVQIIDGNLGDLRDILKKGATFNRETPGVPIAYTTNFLKDNELAVIKNNSEYIETTSKAYTDGKINIDHSGGYVAQFNISWDEVNYDPEGNEIVQHKNWSENNKSKLAHFTSSIYLPGNARNINVYAKECTGLAWEWWRTVIDDRNLPLVKNRNISIWGTTLYPKYSNKVDNPIE

SEQ ID NO: 15 - DNA, 588 bp, Artificial sequence
  source 1..588: mol_type = other DNA
atgggcgcggacgacgttgttgactcttctaaatctttcgttatggaaaacttctcttcttaccacggcaccaaaccgggctacgttgactctatccagaaaggcatccagaaaccgaaatctggcacccagggcaactacgacgacgactggaaaggcttctactctaccgacaacaaatacgacgcggcgggctactctgttgacaacgaaaacccgctgtctggcaaagcgggcggcgttgttaaagttacctacccgggcctgaccaaagttctggcgctgaaagttgacaacgcggaaaccatcaaaaaagaactgggcctgtctctgaccgaaccgctgatggaacaggttggcaccgaagaatttatcaaacgtttcggcgacggcgcgtctcgtgttgttctgtctctgccgttcgcggaaggctcttcttctgttgaatacatcaacaactgggaacaggcgaaagcgctgtctgttgaactggaaatcaacttcgaaacccgtggcaaacgtggccaggacgcgatgtacgaatacatggcgcaggcgtgcgcgggcaaccgtgttcgtcgttcttaa

SEQ ID NO: 16 - protein, 195 aa, Artificial sequence
MGADDVVDSSKSFVMENFSSYHGTKPGYVDSIQKGIQKPKSGTQGNYDDDWKGFYSTDNKYDAAGYSVDNENPLSGKAGGVVKVTYPGLTKVLALKVDNAETIKKELGLSLTEPLMEQVGTEEFIKRFGDGASRVVLSLPFAEGSSSVEYINNWEQAKALSVELEINFETRGKRGQDAMYEYMAQACAGNRVRRS

SEQ ID NO: 17 - DNA, 777 bp, Artificial sequence
  source 1..777: mol_type = other DNA
atggtgaaaatcattttcgtattttttatttttctgagcagcttcagctatgccaacgatgataaactgtaccgcgcggatagccgcccgccggatgaaattaaacagagcggtggtctgatgccgcgcggccagtcggaatactttgatcgcggcacccagatgaacattaacctgtacgaccatgcccgcggcacccagaccggctttgtgcgccatgatgatggctacgtgagcaccagtattagcctgcgcagcgcgcatctggtgggccagaccattctgagcggccattcgacctattatatttatgtgattgcgaccgcgccgaacatgtttaatgtgaatgatgtgctgggcgcctatagcccgcacccggatgaacaggaagtgagcgcgctgggcggcattccgtatagccagatttacggctggtatcgcgtgcactttggcgtcctggatgaacagctgcaccgcaaccgcggctaccgtgatcgctattatagcaacctggatattgcgccggccgcggatggctatggcctggcgggctttcctccggaacatcgcgcgtggcgcgaggaaccgtggattcaccacgccccgccgggctgcggcaacgccccgcgcagcagcatgagcaacacctgcgatgaaaaaacccagagcctgggcgtgaaatttctggatgaataccagtcaaaagtgaaacgccagatctttagcggctatcagagcgatattgatacccataaccgcattaaagatgaactgtga

SEQ ID NO: 18 - protein, 258 aa, Artificial sequence
MVKIIFVFFIFLSSFSYANDDKLYRADSRPPDEIKQSGGLMPRGQSEYFDRGTQMNINLYDHARGTQTGFVRHDDGYVSTSISLRSAHLVGQTILSGHSTYYIYVIATAPNMFNVNDVLGAYSPHPDEQEVSALGGIPYSQIYGWYRVHFGVLDEQLHRNRGYRDRYYSNLDIAPAADGYGLAGFPPEHRAWREEPWIHHAPPGCGNAPRSSMSNTCDEKTQSLGVKFLDEYQSKVKRQIFSGYQSDIDTHNRIKDEL

SEQ ID NO: 19 - DNA, 948 bp, Artificial sequence
  source 1..948: mol_type = other DNA
atgaaaataattatttttagagtgctaacttttttctttgttatcttttcagttaatgtggttgcgaaggaatttaccttagacttctcgactgcaaagacgtatgtagattcgctgaatgtcattcgctctgcaataggtactccattacagactatttcatcaggaggtacgtctttactgatgattgatagtggcacaggggataatttgtttgcagttgatgtcagagggatagatccagaggaagggcggtttaataatctacggcttattgttgaacgaaataatttatatgtgacaggatttgttaacaggacaaataatgttttttatcgctttgctgatttttcacatgttacctttccaggtacaacagcggttacattgtctggtgacagtagctataccacgttacagcgtgttgcagggatcagtcgtacggggatgcagataaatcgccattcgttgactacttcttatctggatttaatgtcgcatagtggaacctcactgacgcagtctgtggcaagagcgatgttacggtttgttactgtgacagctgaagctttacgttttcggcaaatacagaggggatttcgtacaacactggatgatctcagtgggcgttcttatgtaatgactgctgaagatgttgatcttacattgaactggggaaggttgagtagtgtcctgcctgattatcatggacaagactctgttcgtgtaggaagaatttcttttggaagcattaatgcaattctgggaagcgtggcattaatactgaattgtcatcatcatgcatcgcgagttgccagaatggcatctgatgagtttccttctatgtgtccggcagatggaagagtccgtgggattacgcacaataaaatattgtgggattcatccactctgggggcaattctgatgcgcagaactattagcagttga

SEQ ID NO: 20 - protein, 315 aa, Artificial sequence [sequence omitted]

SEQ ID NO: 21 - DNA, 960 bp, Artificial sequence
  source 1..960: mol_type = other DNA
atgaagtgtatattatttaaatgggtactgtgcctgttactgggtttttcttcggtatcctattcccgggagtttacgatagacttttcgacccaacaaagttatgtctcttcgttaaatagtatacggacagagatatcgacccctcttgaacatatatctcaggggaccacatcggtgtctgttattaaccacaccccaccgggcagttattttgctgtggatatacgagggcttgatgtctatcaggcgcgttttgaccatcttcgtctgattattgagcaaaataatttatatgtggccgggttcgttaatacggcaacaaatactttctaccgtttttcagattttacacatatatcagtgcccggtgtgacaacggtttccatgacaacggacagcagttataccactctgcaacgtgtcgcagcgctggaacgttccggaatgcaaatcagtcgtcactcactggtttcatcatatctggcgttaatggagttcagtggtaatacaatgaccagagatgcatccagagcagttctgcgttttgtcactgtcacagcagaagccttacgcttcaggcagatacagagagaatttcgtcaggcactgtctgaaactgctcctgtgtatacgatgacgccgggagacgtggacctcactctgaactgggggcgaatcagcaatgtgcttccggagtatcggggagaggatggtgtcagagtggggagaatatcctttaataatatatcagcgatactggggactgtggccgttatactgaattgccatcatcagggggcgcgttctgttcgcgccgtgaatgaagagagtcaaccagaatgtcagataactggcgacaggcctgttataaaaataaacaatacattatgggaaagtaatacagctgcagcgtttctgaacagaaagtcacagtttttatatacaacgggtaaataa

SEQ ID NO: 22 - protein, 319 aa, Artificial sequence
MKCILFKWVLCLLLGFSSVSYSREFTIDFSTQQSYVSSLNSIRTEISTPLEHISQGTTSVSVINHTPPGSYFAVDIRGLDVYQARFDHLRLIIEQNNLYVAGFVNTATNTFYRFSDFTHISVPGVTTVSMTTDSSYTTLQRVAALERSGMQISRHSLVSSYLALMEFSGNTMTRDASRAVLRFVTVTAEALRFRQIQREFRQALSETAPVYTMTPGDVDLTLNWGRISNVLPEYRGEDGVRVGRISFNNISAILGTVAVILNCHHQGARSVRAVNEESQPECQITGDRPVIKINNTLWESNTAAAFLNRKSQFLYTTGK

SEQ ID NO: 23 - DNA, 711 bp, Artificial sequence
  source 1..711: mol_type = other DNA
atggatgatccgccggccaccgtgtatcgctacgattcgcgcccgccggaagatgtgtttcagaacggctttaccgcctggggcaataacgataatgttctggatcacctgaccggtcgttcatgccaggtgggcagcagcaacagcgccttcgtgagcaccagcagcagccgccgctataccgaagtgtacctggaacatcgcatgcaggaagccgtggaagcggaacgcgcaggccgtggcaccggccactttattggctatatttatgaggtgcgcgccgataacaacttttacggcgccgcatcaagctactttgaatacgtggatacctatggcgataacgcgggccgcattctggcgggcgcgctggcgacctatcagagcgaatatctggcccaccgccgtattccgccggaaaatattcgccgcgttacccgcgtgtatcataatggcattaccggcgaaaccaccaccaccgaatatagcaacgcgcgctatgtgagccagcagacccgcgcgaacccgaacccgtatacctcccgtcgtagcgtggctagcattgtgggtaccctggtgcgcatggcgccggtgattggcgcgtgcatggcgcgtcaggccgaaagcagcgaagcgatggcggcctggagcgaacgcgcgggcgaagcgatggtgctggtgtactacgaatcgattgcctatagcttttaa

SEQ ID NO: 24 - protein, 236 aa, Artificial sequence
MDDPPATVYRYDSRPPEDVFQNGFTAWGNNDNVLDHLTGRSCQVGSSNSAFVSTSSSRRYTEVYLEHRMQEAVEAERAGRGTGHFIGYIYEVRADNNFYGAASSYFEYVDTYGDNAGRILAGALATYQSEYLAHRRIPPENIRRVTRVYHNGITGETTTTEYSNARYVSQQTRANPNPYTSRRSVASIVGTLVRMAPVIGACMARQAESSEAMAAWSERAGEAMVLVYYESIAYSF

SEQ ID NO: 25 - DNA, 1917 bp, Artificial sequence
  source 1..1917: mol_type = other DNA
atgcacctgaccccacattggattccgctggtggcaagcctgggcctgcttgcgggcggcagctttgcgagcgcggccgaagaagcatttgatttgtggaacgaatgtgccaaagcgtgtgtgctggatcttaaagatggcgttcgtagtagccgcatgtcagttgatccggcaatcgcggataccaatggtcagggcgttctgcattattcaatggtgctggaaggcggcaatgatgcgctgaaactggccattgacaatgcactgagcattaccagcgatggcctgaccattcgtctggaaggcggcgtggaaccgaataaaccggtgcgctatagctacacccgccaggcccgtggcagctggagcctgaactggctggtgccgattggccatgaaaaaccgagcaatattaaagtgtttattcacgaattaaacgccggtaaccagctgagccacatgagtccgatttatactattgaaatgggcgatgaactgctggcgaaactggcccgtgatgccaccttcttcgttcgcgcgcatgaaagcaatgaaatgcagccgaccctggcgatttcacacgccggcgtatcagttgtgatggcccaggcgcagcctcgccgcgaaaaacgctggagcgaatgggccagcggtaaagtgctgtgcctgctggatccactggatggcgtgtataattatctggcgcagcagcgttgcaatctggatgatacctgggaaggtaaaatttatcgtgtgctggccggcaatccggcgaaacatgatctggatattaaaccgaccgtgattagccatcgcctgcattttccggaaggcggtagcctggcggccctgaccgcgcatcaggcgtgccatctgccgttggaaacctttacccgccatcgtcagccgcgtggttgggaacagctggaacagtgtggctatccggtgcagcgcctggtggcactgtacctggcggcccgtctgagctggaaccaggttgatcaggttattcgcaatgccctggccagcccgggcagcggcggcgatttaggcgaagctattcgcgaacagccggaacaggcccgcctggccctgaccctggcggcggccgaaagcgaacgctttgtgcgccagggcaccggcaatgatgaagcgggcgcggcgagcgcagatgttgtgagcctgacctgcccggtggcggccggcgaatgtgcgggcccggcggatagcggtgatgccctgctggaacgtaattatccgaccggtgccgaatttctgggcgatggcggcgatatctcgttcagcacccgtggcacgcagaactggacggtcgaacgtctgctgcaagcccatcgccagctggaagaacgcggctatgtattcgtgggctatcatggcacctttctggaagcggcccagagcattgtttttggcggcgtgcgtgcccgttctcaggatctggatgcgatttggcgcggcttttatattgccggtgatcccgcgctggcttatggctacgcacaggatcaggaaccggacgcgcgcggccgtattcgcaacggcgcgctgctgcgtgtgtatgtgccgcgcagcagcctgccgggcttttatcgtacgggcctgaccctggccgccccggaagccgccggcgaagtagaacgtctgattggccatccgctgccgcttcgcctggatgcgattaccggcccggaagaggaaggcggtcgtctggaaacgattctgggctggccgttggcggaacgcaccgtggtgattccgagcgcgattccgaccgatccgcgcaacgttggcggcgacctggacccgtcatcgattccagataaagaacaggcgatcagcgcgctgccggattatgcgtcgcagccgggcaaaccgccgcgcgaagatctgaaataa

SEQ ID NO: 26 - protein, 638 aa, Artificial sequence
MHLTPHWIPLVASLGLLAGGSFASAAEEAFDLWNECAKACVLDLKDGVRSSRMSVDPAIADTNGQGVLHYSMVLEGGNDALKLAIDNALSITSDGLTIRLEGGVEPNKPVRYSYTRQARGSWSLNWLVPIGHEKPSNIKVFIHELNAGNQLSHMSPIYTIEMGDELLAKLARDATFFVRAHESNEMQPTLAISHAGVSVVMAQAQPRREKRWSEWASGKVLCLLDPLDGVYNYLAQQRCNLDDTWEGKIYRVLAGNPAKHDLDIKPTVISHRLHFPEGGSLAALTAHQACHLPLETFTRHRQPRGWEQLEQCGYPVQRLVALYLAARLSWNQVDQVIRNALASPGSGGDLGEAIREQPEQARLALTLAAAESERFVRQGTGNDEAGAASADVVSLTCPVAAGECAGPADSGDALLERNYPTGAEFLGDGGDISFSTRGTQNWTVERLLQAHRQLEERGYVFVGYHGTFLEAAQSIVFGGVRARSQDLDAIWRGFYIAGDPALAYGYAQDQEPDARGRIRNGALLRVYVPRSSLPGFYRTGLTLAAPEAAGEVERLIGHPLPLRLDAITGPEEEGGRLETILGWPLAERTVVIPSAIPTDPRNVGGDLDPSSIPDKEQAISALPDYASQPGKPPREDLK

SEQ ID NO: 27 - DNA, 1080 bp, Artificial sequence
  source 1..1080: mol_type = other DNA
atgcaagcggcaacagtcgtcattaaccgccgcgctctgcgacacaacctgcaacgtctgcgtgaactggcgcctgccagtaagctggttgcggtggtgaaagcgaacgcttatggacacggtcttctggagaccgcgcgaacgctccctgatgctgacgcttttggcgtggcgcgtcttgaagaggctctacgtctgcgagcgggcgggatcacgcagccaatcctgctgctggagggttttttcgacgccgccgatttgccgaccatttccgcgcaatgtctgcataccgccgtacataatcaagagcagcttgccgccctggaggcggtggagctggcggagccggtaacggtctggatgaagctggataccggtatgcatcgtctcggcgtgcgtcccgaagaggcggaggcgttctaccagcgtctgacgcactgtaaaaatgtacgccagccggtgaatatcgtcagccattttgcccgtgcggatgagccggaatgcggcgctaccgaacatcagctcgacatttttaatgccttctgtcagggtaaacccggtcagcgctctattgccgcgtctggcggtatcctgctgtggccgcagtctcactttgactgggcgcgtccgggcatcattttgtatggcgtatcgccgctggagcacaaaccctgggggccggattttggttttcagccggtgatgtccttaacctccagtttgatcgcggtgcgtgaccacaaagcgggcgaaccggtgggctacggcgggacatgggtgagtgagcgcgacacgcgcctgggcgtggtggcgatgggttatggcgatggctacccacgagcggcgccttccggtacgccagtactggtcaatggtcgtgaagttccgattgtcgggcgggtggcgatggatatgatttgcgtagatttggggccaaacgcgcaggataacgcgggcgatccggtggtcttatggggtgaaggtctgccggttgaacgtatcgctgaaatgacaaaagtaagtgcttacgaacttatcacgcgcctgacctcaagggtggcgatgaagtatattgattaa

SEQ ID NO: 28 - protein, 359 aa, Artificial sequence
MQAATVVINRRALRHNLQRLRELAPASKLVAVVKANAYGHGLLETARTLPDADAFGVARLEEALRLRAGGITQPILLLEGFFDAADLPTISAQCLHTAVHNQEQLAALEAVELAEPVTVWMKLDTGMHRLGVRPEEAEAFYQRLTHCKNVRQPVNIVSHFARADEPECGATEHQLDIFNAFCQGKPGQRSIAASGGILLWPQSHFDWARPGIILYGVSPLEHKPWGPDFGFQPVMSLTSSLIAVRDHKAGEPVGYGGTWVSERDTRLGVVAMGYGDGYPRAAPSGTPVLVNGREVPIVGRVAMDMICVDLGPNAQDNAGDPVVLWGEGLPVERIAEMTKVSAYELITRLTSRVAMKYID

SEQ ID NO: 29 - DNA, 1071 bp, Artificial sequence
  source 1..1071: mol_type = other DNA
atgacccgccctatacaggccagccttgatttacaggtaatgaaacaaaatttggctattgtgcgccgggcggccccagaggcgcgcgtctggtcggtagtgaaagccaacgcctacggccacggtattgaacgcgtctggagcgcgctgggcgccacagatggtttcgctatgctcaaccttgaagaggcgattaccctgcgtgagcgcgggtggaaagggccgatattgatgctggaggggtttttccatgcgcaagacctggaggcgtatgacacttatcggctgaccacctgcatccacagtaactggcagttgaaagcgctgcaaaatgcgcggcttaacgcgccgctggatatctatgtcaaagtcaacagcggcatgaaccgactcggttttcagcctgagcgggcgcagaccgtctggcagcaattgcgggcaatgcgcaatgtcggtgaaatgaccctgatgtcacattttgctcaggccgatcatccggaaggtatcggggaggcgatgaggcgtattgcgctggcgacggaaggtcttcagtgtgcatactcgttatcaaattcggcagcgacgctgtggcatccccaggcgcattatgactgggtcaggccgggcattattttgtacggcgcgtcgccgtcaggacagtggcgggatattgccgataccggactaaaacctgtgatgacgctgagtagcgaaattattggcgtgcagacgctgagcgcgggtgaaagggtaggctatggcggagggtattctgtgactcaggaacaacgcattggcatcgtcgcggcgggttatgccgatggctatccacgccatgcgccgaccgggacgcctgtgctggtggacggtatccgtaccagaacagtaggcaccgtttcaatggatatgctggcggtggatttgacgccgtgtccgcaggcgggaatcggcacgccggttgaattatggggcaaagaaattaaggtcgatgatgtcgcttctgcggcaggcacgctgggctatgagctactgtgcgccgtagcgccgcgtgtgccgtttgtgacaacgtaa

SEQ ID NO: 30 - protein, 356 aa, Artificial sequence
MTRPIQASLDLQVMKQNLAIVRRAAPEARVWSVVKANAYGHGIERVWSALGATDGFAMLNLEEAITLRERGWKGPILMLEGFFHAQDLEAYDTYRLTTCIHSNWQLKALQNARLNAPLDIYVKVNSGMNRLGFQPERAQTVWQQLRAMRNVGEMTLMSHFAQADHPEGIGEAMRRIALATEGLQCAYSLSNSAATLWHPQAHYDWVRPGIILYGASPSGQWRDIADTGLKPVMTLSSEIIGVQTLSAGERVGYGGGYSVTQEQRIGIVAAGYADGYPRHAPTGTPVLVDGIRTRTVGTVSMDMLAVDLTPCPQAGIGTPVELWGKEIKVDDVASAAGTLGYELLCAVAPRVPFVTT

SEQ ID NO: 31 - DNA, 237 bp, Artificial sequence
  source 1..237: mol_type = other DNA
gcgtgaacgcagtttatctaacacgagctttactccctgtttcaatagtcctgttattttgccatatccaataaatcacatggcggcgtaaatcaacaattgggtctgattttctaccccattattggtgttaccaatacgcctttaactgccttaaatcaaaaattgtcgcagcaaggttaactaaaatccctgttcgttaacaattttgcgtctcagacgtaaccctcaggataa

SEQ ID NO: 32 - DNA, 185 bp, Artificial sequence
  source 1..185: mol_type = other DNA
cgctgcactggtaaaagacgcgatgtataacggttctttgttgattcgtctgttgcagggttaacattttttaactgttctaccaaaatttgcgctatctcaatttgggccaggaaagcataacttagactttcaaggttaattattttcctggtttatatttgtgaagcataacggtggagtta

SEQ ID NO: 33 - DNA, 370 bp, Artificial sequence
  source 1..370: mol_type = other DNA
aacattatttgccgttgtaataacgacccggaattataacggctaaataaccatcaattgataaaaaatatatttgtctttttgtgcgcaacagaattttggaaattattggtaatttctacgctacctattttctttacacgattcagccgattaaatttaaatttctgccgttgattgtccttttattgataataaattgttaagtaattgttttatttttacattggttataccaattatccctcaacatcccacttacagacctcatccgttataacgcaaagtttcaacagtgtcttaaagttatttcgacatacttggcaacatatgtgacatgcgcggcagaacttggtaacacagaaccaat

SEQ ID NO: 34 - DNA, 292 bp, Artificial sequence
  source 1..292: mol_type = other DNA
aatgtcatgcctccagtgaatgttacctggagtgtagaaaacctcatccattccggggagaagaatttataaagtgtgatccgacctgaattcattatgcagaacggattgacatgagctggcatatccccgaccagatcgcggcttaacacgcttaacggcagttgaatcatcagtaaaataaaacagttgtaacttgaaatggtaaaatgttaataatattttgctatcaggttatcaaaaacaaacaactttacttgtcacccgcacggctctgtttttaacatcgctt

SEQ ID NO: 35 - DNA, 21 bp, Artificial sequence
  source 1..21: mol_type = other DNA
tagtaagaaggagatatacat

SEQ ID NO: 36 - DNA, 819 bp, Artificial sequence
  source 1..819: mol_type = other DNA
ctcgagcatgtgagcaaaaggccagcaaaaggccaggaaccgtaaaaaggccgcgttgctggcgtttttccataggctccgcccccctgacgagcatcacaaaaatcgacgctcaagtcagaggtggcgaaacccgacaggactataaagataccaggcgtttccccctggaagctccctcgtgcgctctcctgttccgaccctgccgcttaccggatacctgtccgcctttctcccttcgggaagcgtggcgctttctcatagctcacgctgtaggtatctcagttcggtgtaggtcgttcgctccaagctgggctgtgtgcacgaaccccccgttcagcccgaccgctgcgccttatccggtaactatcgtcttgagtccaacccggtaagacacgacttatcgccactggcagcagccactggtaacaggattagcagagcgaggtatgtaggcggtgctacagagttcttgaagtggtggcctaactacggctacactagaaggacagtatttggtatctgcgctctgctgaagccagttaccttcggaaaaagagttggtagctcttgatccggcaaacaaaccaccgctggtagcggtggtttttttgtttgcaagcagcagattacgcgcagaaaaaaaggatctcaagaagatcctttgatcttttctacggggtctgacgctcagtggaacgaaaactcacgttaagggattttggtcatgagattatcaaaaaggatcttcacctagatccttttaaattaaaaatgaagttttaaatcaatctaaagtatatatgagtaagcggccgc

SEQ ID NO: 37 - DNA, 1133 bp, Artificial sequence
  source 1..1133: mol_type = other DNA
actagtgaacctcttcgagggacctaataacttcgtatagcatacattatacgaagttatattaagggttccggatcctaattgatatctaagggcaccaataactgccttaaaaaaattatgcaccaccttgccattcatcacaatactgttgcagttcattcagcatacgaccaacatgaaaaccatcacaaactgcatgatgaacctgaattgccagcggcatcagaactttatcaccctgggtgtaatatttgcccatcgtaaaaaccggtgcgaaaaagttatccatattggccacattcagatcaaatgaggtaaagctaacccacggatttgcgctaacaaagaacatgttttcgataaagcctttcggaaaatatgccaggttttcaccataacatgcaacatcctggctatagatgtgcaggaactgacgaaaatcatcatgatattctgaccacaggctgctaaaggtttcggtctgttcatgaaaaacggtataacacggatgaacgctatcccaaataaccagttcaccatctttcattgccatacgaaattccggatgggcattcatcagacgtgccagaatatgaataaaggcagggtagaacttgtgtttgttctttttcacggttttcagaaatgcggttatatccagctgaacggtctgattataggtacactgtgcaacgctctgaaatgcttcaaagtgttctttacgatgccactggctaatatcaacggtggtataaccggtgattttcttttccattttagcttccttagctcctgaaaatctcgataactcaaaaaatacgcccggtagtgatcttatttcattatggtgaaagttggaacctcttacgtgccgatcaacgtctcattttcgccaaaagttggcccagggcttcccggtatcaacagggacaccaggatttatttattctgcgaagtgatcttccgtcacaggtatttattcggcgcaaagtgcgtcgggtgatgctgccgatatcggacccgggatcctaattggctggacgtaaactcctcttcagacctaataacttcgtatagcatacattatacgaagttatattaagggttattgaatatgatcgggcggccgc

SEQ ID NO: 38 - DNA, 3650 bp, Artificial sequence
  source 1..3650: mol_type = other DNA
gaattctcagccaaacgtctcttcaggccactgactagcgataactttccccacaacggaacaactctcattgcatgggatcattgggtactgtgggtttagtggttgtaaaaacacctgaccgctatccctgatcagtttcttgaaggtaaactcatcacccccaagtctggctatgcagaaatcacctggctcaacagcctgctcagggtcaacgagaattaacattccgtcaggaaagcttggcttggagcctgttggtgcggtcatggaattaccttcaacctcaagccagaatgcagaatcactggcttttttggttgtgcttacccatctctccgcatcacctttggtaaaggttctaagcttaggtgagaacatccctgcctgaacatgagaaaaaacagggtactcatactcacttctaagtgacggctgcatactaaccgcttcatacatctcgtagatttctctggcgattgaagggctaaattcttcaacgctaactttgagaatttttgtaagcaatgcggcgttataagcatttaatgcattgatgccattaaataaagcaccaacgcctgactgccccatccccatcttgtctgcgacagattcctgggataagccaagttcatttttctttttttcataaattgctttaaggcgacgtgcgtcctcaagctgctcttgtgttaatggtttcttttttgtgctcatacgttaaatctatcaccgcaagggataaatatctaacaccgtgcgtgttgactattttacctctggcggtgataatggttgcatgtactaaggaggttgcgcatgcaggtaccaatgtccaatttactgaccgtacaccaaaatttgcctgcattaccggtcgatgcaacgagtgatgaggttcgcaagaacctgatggacatgttcagggatcgccaggcgttttctgagcatacctggaaaatgcttctgtccgtttgccggtcgtgggcggcatggtgcaagttgaataaccggaaatggtttcccgcagaacctgaagatgttcgcgattatcttctatatcttcaggcgcgcggtctggcagtaaaaactatccagcaacatttgggccagctaaacatgcttcatcgtcggtccgggctgccacgaccaagtgacagcaatgctgtttcactggttatgcggcggatccgaaaagaaaacgttgatgccggtgaacgtgcaaaacaggctctagcgttcgaacgcactgatttcgaccaggttcgttcactcatggaaaatagcgatcgctgccaggatatacgtaatctggcatttctggggattgcttataacaccctgttacgtatagccgaaattgccaggatcagggttaaagatatctcacgtactgacggtgggagaatgttaatccatattggcagaacgaaaacgctggttagcaccgcaggtgtagagaaggcacttagcctgggggtaactaaactggtcgagcgatggatttccgtctctggtgtagctgatgatccgaataactacctgttttgccgggtcagaaaaaatggtgttgccgcgccatctgccaccagccagctatcaactcgcgccctggaagggatttttgaagcaactcatcgattgatttacggcgctaaggatgactctggtcagagatacctggcctggtctggacacagtgcccgtgtcggagccgcgcgagatatggcccgcgctggagtttcaataccggagatcatgcaagctggtggctggaccaatgtaaatattgtcatgaactatatccgtaacctggatagtgaaacaggggcaatggtgcgcctgctggaagatggcgattaggggtaccgagctcatgaacgcttattacattcaggatcgtcttgaggctcagagctgggcgcgtcactaccagcagctcgcccgtgaagagaaagaggcagaactggcagacgacatggaaaaaggcctgccccagcacctgtttgaatcgctatgcatcgatcatttgcaacgccacggggccagcaaaaaatccattacccgtgcgtttgatgacgatgttgagtttcaggagcgcatggcagaacacatccggtacatggttgaaaccattgctcaccaccaggttgatattgattcagaggtataaaacgaatgagtactgcactcgcaacgctggctgggaagctggctgaacgtgtcggcatggattctgtcgacccacaggaactgatcaccactcttcgccagacggcatttaaaggtgatgccagcgatgcgcagttcatcgcattactgatcgttgccaaccagtacggccttaatccgtggacgaaagaaatttacgcctttcctgataagcagaatggcatcgttccggtggtgggcgttgatggctggtcccgcatcatcaatgaaaaccagcagtttgatggcatggactttgagcaggacaatgaatcctgtacatgccggatttaccgcaaggaccgtaatcatccgatctgcgttaccgaatggatggatgaatgccgccgcgaaccattcaaaactcgcgaaggcagagaaatcacggggccgtggcagtcgcatcccaaacggatgttacgtcataaagccatgattcagtgtgcccgtctggccttcggatttgctggtatctatgacaaggatgaagccgagcgcattgtcgaaaatactgcatacactgcagaacgtcagccggaacgcgacatcactccggttaacgatgaaaccatgcaggagattaacactctgctgatcgccctggataaaacatgggatgacgacttattgccgctctgttcccagatatttcgccgcgacattcgtgcatcgtcagaactgacacaggccgaagcagtaaaagctcttggattcctgaaacagaaagccgcagagcagaaggtggcagcatgacaccggacattatcctgcagcgtaccgggatcgatgtgagagctgtcgaacagggggatgatgcgtggcacaaattacggctcggcgtcatcaccgcttcagaagttcacaacgtgatagcaaaaccccgctccggaaagaagtggcctgacatgaaaatgtcctacttccacaccctgcttgctgaggtttgcaccggtgtggctccggaagttaacgctaaagcactggcctggggaaaacagtacgagaacgacgccagaaccctgtttgagttcacttccggcgtgaatgttactgaatccccgatcatctatcgcgacgaaagtatgcgtaccgcctgctctcccgatggtttatgcagtgacggcaacggccttgaactgaaatgcccgtttacctcccgggatttcatgaagttccggctcggtggtttcgaggccataaagtcagcttacatggcccaggtgcagtacagcatgtgggtgacgcgaaaaaatgcctggtactttgccaactatgacccgcgtatgaagcgtgaaggcctgcattatgtcgtgattgagcgggatgaaaagtacatggcgagttttgacgagatcgtgccggagttcatcgaaaaaatggacgaggcactggctgaaattggttttgtatttggggagcaatggcgatgactcgag

SEQ ID NO: 39 - DNA, 1147 bp, Artificial sequence
  source 1..1147: mol_type = other DNA
gcggccgcgactagtgaacctcttcgagggacctaataacttcgtatagcatacattatacgaagttatattaagggttccggatcctaagcttgatatctaagggcaccaataactgccttaaaaaaattacgccccgccctgccactcatcgcagtactgttgtaattcattaagcattctgccgacatggaagccatcacagacggcatgatgaacctgaatcgccagcggcatcagcaccttgtcgccttgcgtataatatttgcccatggtgaaaacgggggcgaagaagttgtccatattggccacgtttaaatcaaaactggtgaaactcacccagggattggctgagacgaaaaacatattctcaataaaccctttagggaaataggccaggttttcaccgtaacacgccacatcttgcgaatatatgtgtagaaactgccggaaatcgtcgtggtattcactccagagcgatgaaaacgtttcagtttgctcatggaaaacggtgtaacaagggtgaacactatcccatatcaccagctcaccgtctttcattgccatacggaattccggatgagcattcatcaggcgggcaagaatgtgaataaaggccggataaaacttgtgcttatttttctttacggtctttaaaaaggccgtaatatccagctgaacggtctggttataggtacattgagcaactgactgaaatgcctcaaaatgttctttacgatgccattgggatatatcaacggtggtatatccagtgatttttttctccattttagcttccttagctcctgaaaatctcgataactcaaaaaatacgcccggtagtgatcttatttcattatggtgaaagttggaacctcttacgtgccgatcaacgtctcattttcgccaaaagttggcccagggcttcccggtatcaacagggacaccaggatttatttattctgcgaagtgatcttccgtcacaggtatttattcggcgcaaagtgcgtcgggtgatgctgccgatatcggtacccgggatcctaagcttggctggacgtaaactcctcttcagacctaataacttcgtatagcatacattatacgaagttatattaagggttattgaatatgatcgggcggccgc

SEQ ID NO: 40 - DNA, 428 bp, Artificial sequence
  source 1..428: mol_type = other DNA
gcggccgcaagagaacaacggcaagttacaggatccgcagcaatatcagcaaaacaccttattgcttgaagcgatcgagcaggccgaaaatatcatcaacattatttattatcgttaccataacagcgcacttgtagtgagtgagcaagagtaaagtaaaaatatcttagagcctatcccaccaggcgttaattggcgcagccagtttggacacggatagcgcgcaaaaaccgcagcgtacacgtagtacgtgaggtttgactcgctacgctcgcccttcgggccgccgctagcggcgttcaaaacgctaacgcgttttggcgagcactgcccaggttcaaaatggcaagtaaaatagccctaatgggataggctcttagttagcacgttaattatctatcgaagcttaagaaggagatatacatatg

SEQ ID NO: 41 - DNA, 71 bp, Artificial sequence
  source 1..71: mol_type = other DNA
atggaatccctgacgttacaacccatcgcgcgggtcgatggcgccattaaccgatcatattcaataaccct

SEQ ID NO: 42 - DNA, 72 bp, Artificial sequence
  source 1..72: mol_type = other DNA
gaagacttaggcaggcgtactcattcgcgccagttgttcgaaataatcaggactagtgaacctcttcgaggg

SEQ ID NO: 43 - DNA, 20 bp, Artificial sequence
  source 1..20: mol_type = other DNA
cggacaatacgctggacaag

SEQ ID NO: 44 - DNA, 20 bp, Artificial sequence
  source 1..20: mol_type = other DNA
gcggctttgtaggttgacat

SEQ ID NO: 45 - DNA, 22 bp, Artificial sequence
  source 1..22: mol_type = other DNA
tccttagctcctgaaaatctcg

SEQ ID NO: 46 - DNA, 20 bp, Artificial sequence
  source 1..20: mol_type = other DNA
tgtggcgtgttacggtgaaa

SEQ ID NO: 47 - DNA, 37 bp, Artificial sequence
  source 1..37: mol_type = other DNA
atttgcggccgcgcgtgaacgcagtttatctaacacg

SEQ ID NO: 48 - DNA, 35 bp, Artificial sequence
  source 1..35: mol_type = other DNA
cccaagcttttatcctgagggttacgtctgagacg

SEQ ID NO: 49 - DNA, 32 bp, Artificial sequence
  source 1..32: mol_type = other DNA
atttgcggccgccgctgcactggtaaaagacg

SEQ ID NO: 50 - DNA, 30 bp, Artificial sequence
  source 1..30: mol_type = other DNA
cccaagcttaactccaccgttatgcttcac

SEQ ID NO: 51 - DNA, 43 bp, Artificial sequence
  source 1..43: mol_type = other DNA
cccaagctttggagcgaaaccgatgcaagcggcaacagtcgtc

SEQ ID NO: 52 - DNA, 38 bp, Artificial sequence
  source 1..38: mol_type = other DNA
ccgctcgagttaatcaatatacttcatcgccacccttg

SEQ ID NO: 53 - DNA, 42 bp, Artificial sequence
  source 1..42: mol_type = other DNA
cccaagctttggagcgaaaccgatgacccgccctatacaggc

SEQ ID NO: 54 - DNA, 30 bp, Artificial sequence
  source 1..30: mol_type = other DNA
cccaagcttttacgttgtcacaaacggcac

SEQ ID NO: 55 - DNA, 35 bp, Artificial sequence
  source 1..35: mol_type = other DNA
ccgctcgagattggttctgtgttaccaagttctgc

SEQ ID NO: 56 - DNA, 35 bp, Artificial sequence
  source 1..35: mol_type = other DNA
aaaactgcagaacattatttgccgttgtaataacg

SEQ ID NO: 57 - DNA, 32 bp, Artificial sequence
  source 1..32: mol_type = other DNA
ccgctcgagaagcgatgttaaaaacagagccg

SEQ ID NO: 58 - DNA, 36 bp, Artificial sequence
  source 1..36: mol_type = other DNA
aaaactgcagaatgtcatgcctccagtgaatgttac

SEQ ID NO: 59 - DNA, 20 bp, Artificial sequence
  source 1..20: mol_type = other DNA
ggtacgcaagattggggtac

SEQ ID NO: 60 - DNA, 20 bp, Artificial sequence
  source 1..20: mol_type = other DNA
tgtcagctctttacccagcg

SEQ ID NO: 61 - DNA, 71 bp, Artificial sequence
  source 1..71: mol_type = other DNA
gcaatacgatgatgagtaactctccgtcattcttttaacaaggaattcaaccgatcatattcaataaccct

SEQ ID NO: 62 - DNA, 72 bp, Artificial sequence
  source 1..72: mol_type = other DNA
tgcgcgatacaagccggataagcgcaagcgccacccggcccgccgcgtatgactagtgaacctcttcgaggg

SEQ ID NO: 63 - DNA, 20 bp, Artificial sequence
  source 1..20: mol_type = other DNA
caggtcttacgccgacagaa

SEQ ID NO: 64 - DNA, 20 bp, Artificial sequence
  source 1..20: mol_type = other DNA
gttgctgaagaaccgggtga

SEQ ID NO: 65 - DNA, 20 bp, Artificial sequence
  source 1..20: mol_type = other DNA
cgacggcgatgcttaaaggc

SEQ ID NO: 66 - DNA, 67 bp, Artificial sequence
  source 1..67: mol_type = other DNA
cacccccccgcaacgtttgcatagcgcgcataactgataaaggaagtgaacaggaaacagctatgac

SEQ ID NO: 67 - DNA, 67 bp, Artificial sequence
  source 1..67: mol_type = other DNA
acgtcgacccgcccccaagtggaccggtcgacgccttagcctgaattagggtaaaacgacggccagt

SEQ ID NO: 68 - DNA, 70 bp, Artificial sequence
  source 1..70: mol_type = other DNA
gcaatacgatgatgagtaactctccgtcattcttttaacaaggaattcaagaacaggaaacagctatgac

SEQ ID NO: 69 - DNA, 67 bp, Artificial sequence
  source 1..67: mol_type = other DNA
tgcgcgatacaagccggataagcgcaagcgccacccggcccgccgcgtatgtaaaacgacggccagt

SEQ ID NO: 70 - DNA, 20 bp, Artificial sequence
  source 1..20: mol_type = other DNA
gcaccttaggctggacgatg

SEQ ID NO: 71 - DNA, 20 bp, Artificial sequence
  source 1..20: mol_type = other DNA
taaccgctccctggaacaac

SEQ ID NO: 72 - DNA, 20 bp, Artificial sequence
  source 1..20: mol_type = other DNA
ggtaagcaacgtaacggtcc

SEQ ID NO: 73 - DNA, 67 bp, Artificial sequence
  source 1..67: mol_type = other DNA
ggccgctcactcattaggcaccccaggctttacactttatgcttccggctcgtataatgtgtggaaa

SEQ ID NO: 74 - DNA, 67 bp, Artificial sequence
  source 1..67: mol_type = other DNA
agcttttccacacattatacgagccggaagcataaagtgtaaagcctggggtgcctaatgagtgagc

SEQ ID NO: 75 - DNA, 58 bp, Artificial sequence
  source 1..58: mol_type = other DNA
cgcatacacagcacatctctttgcaggaaaaaaacgctgaacaggaaacagctatgac

SEQ ID NO: 76 - DNA, 54 bp, Artificial sequence
  source 1..54: mol_type = other DNA
gaaccacacgcaggcccgataagcgctgcaatagccagtaaaacgacggccagt

SEQ ID NO: 77 - DNA, 20 bp, Artificial sequence
  source 1..20: mol_type = other DNA
gactgccgattgccattacc

SEQ ID NO: 78 - DNA, 20 bp, Artificial sequence
  source 1..20: mol_type = other DNA
tgaggttctgctgtccgtgc

SEQ ID NO: 79 - DNA, 22 bp, Artificial sequence
  source 1..22: mol_type = other DNA
catatctgcttcaacaacctgc

SEQ ID NO: 80 - DNA, 20 bp, Artificial sequence
  source 1..20: mol_type = other DNA
cgtgaagaactgccgatgaa

SEQ ID NO: 81 - DNA, 20 bp, Artificial sequence
  source 1..20: mol_type = other DNA
atcgtcttgagtccaacccg

SEQ ID NO: 82 - DNA, 20 bp, Artificial sequence
  source 1..20: mol_type = other DNA
ttcgttgccgtctttgtagc

SEQ ID NO: 83 - DNA, 25 bp, Artificial sequence
  source 1..25: mol_type = other DNA
aatacgactcactatagggagagct

SEQ ID NO: 84 - DNA, 20 bp, Artificial sequence
  source 1..20: mol_type = other DNA
tacgccatttcgtcgtcgta

SEQ ID NO: 85 - DNA, 20 bp, Artificial sequence
  source 1..20: mol_type = other DNA
accctgtctatcgacctgcc

SEQ ID NO: 86 - DNA, 20 bp, Artificial sequence
  source 1..20: mol_type = other DNA
aacagatttgccgcttaccg

SEQ ID NO: 87 - DNA, 20 bp, Artificial sequence
  source 1..20: mol_type = other DNA
acccgtccgtctcgtttctt

SEQ ID NO: 88 - DNA, 20 bp, Artificial sequence
  source 1..20: mol_type = other DNA
cgatcgggttgtcaactttg

SEQ ID NO: 89 - DNA, 20 bp, Artificial sequence
  source 1..20: mol_type = other DNA
gaatggtggcgtaccgttat

SEQ ID NO: 90 - DNA, 20 bp, Artificial sequence
  source 1..20: mol_type = other DNA
accgacaacaaatacgacgc

SEQ ID NO: 91 - DNA, 20 bp, Artificial sequence
  source 1..20: mol_type = other DNA
tacggtaaacgccgacaaga

SEQ ID NO: 92 - DNA, 20 bp, Artificial sequence
  source 1..20: mol_type = other DNA
aaaacagggcgaatagcgtc

SEQ ID NO: 93 - DNA, 20 bp, Artificial sequence
  source 1..20: mol_type = other DNA
acttgcgactttggctgctt

SEQ ID NO: 94 - DNA, 20 bp, Artificial sequence
  source 1..20: mol_type = other DNA
cgggtcaatgccgtaacttt

SEQ ID NO: 95 - DNA, 20 bp, Artificial sequence
  source 1..20: mol_type = other DNA
gcctgatgttgatgtcgctg

SEQ ID NO: 96 - DNA, 20 bp, Artificial sequence
  source 1..20: mol_type = other DNA
tacggtaaacgccgacaaga

SEQ ID NO: 97 - DNA, 20 bp, Artificial sequence
  source 1..20: mol_type = other DNA
cataatccgtgggcgaaagt

SEQ ID NO: 98 - DNA, 20 bp, Artificial sequence
  source 1..20: mol_type = other DNA
taccagcggtggtttgtttg

SEQ ID NO: 99 - DNA, 31 bp, Artificial sequence
  source 1..31: mol_type = other DNA
aaactgcagaagagaacaacggcaagttaca

SEQ ID NO: 100 - DNA, 36 bp, Artificial sequence
  source 1..36: mol_type = other DNA
gggaattccatatgtatatctccttcttaagcttcg

SEQ ID NO: 101 - DNA, 20 bp, Artificial sequence
  source 1..20: mol_type = other DNA
tgacgctcagtggaacgaaa